European Patent Specification EP 3 893 841 B1, published April 15, 2026. Title: ANTIBODY FORMULATIONS. Applicant: MORPHOSYS AG. The sequence listing filed with the application follows.

SEQUENCE LISTING (11 sequences)

SEQ ID NO: 1 - protein, 5 aa, Artificial Sequence
  source: /note="Description of Artificial Sequence: Synthetic peptide"
SYYMN

SEQ ID NO: 2 - protein, 17 aa, Artificial Sequence
  source: /note="Description of Artificial Sequence: Synthetic peptide"
GISGDPSNTYYADSVKG

SEQ ID NO: 3 - protein, 11 aa, Artificial Sequence
  source: /note="Description of Artificial Sequence: Synthetic peptide"
DLPLVYTGFAY

SEQ ID NO: 4 - protein, 11 aa, Artificial Sequence
  source: /note="Description of Artificial Sequence: Synthetic peptide"
SGDNLRHYYVY

SEQ ID NO: 5 - protein, 7 aa, Artificial Sequence
  source: /note="Description of Artificial Sequence: Synthetic peptide"
GDSKRPS

SEQ ID NO: 6 - protein, 9 aa, Artificial Sequence
  source: /note="Description of Artificial Sequence: Synthetic peptide"
QTYTGGASL

SEQ ID NO: 7 - protein, 120 aa, Artificial Sequence
  source: /note="Description of Artificial Sequence: Synthetic polypeptide"
QVQLVESGGGLVQPGGSLRLSCAASGFTFSSYYMNWVRQAPGKGLEWVSGISGDPSNTYYADSVKGRFTISRDNSKNTLYLQMNSLRAEDTAVYYCARDLPLVYTGFAYWGQGTLVTVSS

SEQ ID NO: 8 - protein, 109 aa, Artificial Sequence
  source: /note="Description of Artificial Sequence: Synthetic polypeptide"
DIELTQPPSVSVAPGQTARISCSGDNLRHYYVYWYQQKPGQAPVLVIYGDSKRPSGIPERFSGSNSGNTATLTISGTQAEDEADYYCQTYTGGASLVFGGGTKLTVLGQ

SEQ ID NO: 9 - protein, 300 aa, Homo sapiens
MANCEFSPVSGDKPCCRLSRRAQLCLGVSILVLILVVVLAVVVPRWRQQWSGPGTTKRFPETVLARCVKYTEIHPEMRHVDCQSVWDAFKGAFISKHPCNITEEDYQPLMKLGTQTVPCNKILLWSRIKDLAHQFTQVQRDMFTLEDTLLGYLADDLTWCGEFNTSKINYQSCPDWRKDCSNNPVSVFWKTVSRRFAEAACDVVHVMLNGSRSKIFDKNSTFGSVEVHNLQPEKVQTLEAWVIHGGREDSRDLCQDPTIKELESIISKRNIQFSCKNIYRPDKFLQCVKNPEDSSCTSEI

SEQ ID NO: 10 - DNA, 360 bp, Artificial Sequence
  source: /note="Description of Artificial Sequence: Synthetic polynucleotide"
caggtgcaattggtggaaagcggcggcggcctggtgcaaccgggcggcagcctgcgtctgagctgcgcggcctccggatttaccttttcttcttattatatgaattgggtgcgccaagcccctgggaagggtctcgagtgggtgagcggtatctctggtgatcctagcaatacctattatgcggatagcgtgaaaggccgttttaccatttcacgtgataattcgaaaaacaccctgtatctgcaaatgaacagcctgcgtgcggaagatacggccgtgtattattgcgcgcgtgatcttcctcttgtttatactggttttgcttattggggccaaggcaccctggtgacggttagctca

SEQ ID NO: 11 - DNA, 327 bp, Artificial Sequence
  source: /note="Description of Artificial Sequence: Synthetic polynucleotide"
gatatcgaactgacccagccgccttcagtgagcgttgcaccaggtcagaccgcgcgtatctcgtgtagcggcgataatcttcgtcattattatgtttattggtaccagcagaaacccgggcaggcgccagttcttgtgatttatggtgattctaagcgtccctcaggcatcccggaacgctttagcggatccaacagcggcaacaccgcgaccctgaccattagcggcactcaggcggaagacgaagcggattattattgccagacttatactggtggtgcttctcttgtgtttggcggcggcacgaagttaaccgttcttggccag